European Patent Application EP 4 148 063 A1, published March 15, 2023. Title: Engineered spider silk proteins and uses thereof. Applicant: Spiber Technologies AB. Application EP. The sequence listing filed with the application follows.

SEQUENCE LISTING (79 sequences)

SEQ ID NO: 1 - protein, 137 aa, Euprosthenops australis
  VARIANT 6: note = deletion (deltaHis)
GSGNSHTTPWTNPGLAENFMNSFMQGLSSMPGFTASQLDDMSTIAQSMVQSIQSLAAQGRTSPNKLQALNMAFASSMAEIAASEEGGGSLSTKTSSIASAMSNAFLQTTGVVNQPFINEITQLVSMFAQAGMNDVSA

SEQ ID NO: 2 - protein, 131 aa, synthetic construct
  source 1..131: note = Consensus sequence derived from spidroin NT fragments
  REGION 1..131: note = Consensus sequence derived from spidroin NT fragments
  VARIANT 20: note = Leu
  VARIANT 42: note = Asn
  VARIANT 42: note = Gln
  VARIANT 50: note = Ser
  VARIANT 50: note = Lys
  VARIANT 56: note = Arg
  VARIANT 84: note = Leu
  VARIANT 114: note = Ser
  VARIANT 121: note = Asn
  VARIANT 123: note = Leu
  VARIANT 124: note = Ser
QANTPWSSPNLADAFINSFMSAASSSGAFSADQLDDMSTIGDTLMSAMDNMGRSGKSTKSKLQALNMAFASSMAEIAAAESGGGSVGVKTNAISDALSSAFYQTTGSVNPQFVNEIRSLIGMFAQASANEV

SEQ ID NO: 3 - protein, 1110 aa, Euprosthenops australis
  REPEAT 7..19
  REPEAT 20..42
  REPEAT 43..56
  REPEAT 57..70
  REPEAT 71..83
  REPEAT 84..106
  REPEAT 107..120
  REPEAT 121..134
  REPEAT 135..147
  REPEAT 148..170
  REPEAT 171..183
  REPEAT 184..197
  REPEAT 198..211
  REPEAT 212..234
  REPEAT 235..248
  REPEAT 249..265
  REPEAT 266..279
  REPEAT 280..293
  REPEAT 294..306
  REPEAT 307..329
  REPEAT 330..342
  REPEAT 343..356
  REPEAT 357..370
  REPEAT 371..393
  REPEAT 394..406
  REPEAT 407..420
  REPEAT 421..434
  REPEAT 435..457
  REPEAT 458..470
  REPEAT 471..488
  REPEAT 489..502
  REPEAT 503..516
  REPEAT 517..529
  REPEAT 530..552
  REPEAT 553..566
  REPEAT 567..580
  REPEAT 581..594
  REPEAT 595..617
  REPEAT 618..630
  REPEAT 631..647
  REPEAT 648..661
  REPEAT 662..675
  REPEAT 676..688
  REPEAT 689..711
  REPEAT 712..725
  REPEAT 726..739
  REPEAT 740..752
  REPEAT 753..775
  REPEAT 776..789
  REPEAT 790..803
  REPEAT 804..816
  REPEAT 817..839
  REPEAT 840..853
  REPEAT 854..867
  REPEAT 868..880
  REPEAT 881..903
  REPEAT 904..917
  REPEAT 918..931
  REPEAT 932..945
  REPEAT 946..968
  REPEAT 969..981
  REPEAT 982..998
  REPEAT 999..1013
  REPEAT 1014..1027
  REPEAT 1028..1042
  REPEAT 1043..1059
  REPEAT 1060..1073
  REPEAT 1074..1092
QGAGGNAAAAAAAAAAAAAGQGGQGGYGGLGQGGYGQGAGSSAAAAAAAAAAAAAAGRGQGGYGQGSGGNAAAAAAAAAAAASGQGGQGGQGGQGQGGYGQGAGSSAAAAAAAAAAAAAAGQGQGRYGQGAGGNAAAAAAAAAAAAAGQGGQGGQGGLGQGGYGQGAGSSAAAAAASAAAAAAGRGQGGYGQGAGGNAAAAAAAAAAAAAAGQGGQGGYGGLGQGGYGQGAGSSAAAAAAAAAAAAAGGQGGQGQGRYGQGAGSSAAAAAAAAAAAAAAGQGQGGYGQGAGGNAAAAAAAAAAAAAGQGGQGGQGGLGQGGYGQGAGSSAAAAAAAAAAAAAGRGQGGYGQGAGGNAAAAAAAAAEAAAAGQGGQGGYGGLGQGGYGQGAGSSAAAAAAAAAAAAAGRGQGGYGQGAGGNAAAAAAAAAAAAAAGQGGQGGYGGLGQGGYGQGAGSSAAAAAAAAAAAAAGGQGGQGQGRYGQGAGSSAAAAAAAAAAAAAAGRGQGGYGQGSGGNAAAAAAAAAAAASGQGSQGGQGGQGQGGYGQGAGSSAAAAAAAAAAAAASGRGQGGYGQGAGGNAAAAAAAAAAAAAAGQGGQGGYGGLGQGGYGQGAGSSAAAAAAAAAAAAGGQGGQGQGGYGQGAGSSAAAAAAAAAAAAAAGRGQGGYGQGSGGNAAAAAAAAAAAASGQGGQGGQGGQGQGGYGQGAGSSAAAAAAAAAAAAAAGQGQGGYGQGAGGNAAAAAAAAAAAAAGQGGQGGQGGLGQGGYGQGAGSSAAAAAAAAAAAAAAGRGQGGYGQGVGGNAAAAAAAAAAAAAGQGGQGGQGGLGQGGYGQGAGSSAAAAAAAAAAAAAAGRGQGGYGQGSGGNAAAAAAAAAAAASGQGSQGGQGGQGQGGYGQGAGSSAAAAAAAAAAAAASGRGQGGYGQGAGGNAAAAAAAAAAAAAAGQGGQGGYGGLGQGGYGQGAGSSAAAAAAAAAAAAGGQGGQGQGGYGQGSGGSAAAAAAAAAAAAAAAGRGQGGYGQGSGGNAAAAAAAAAAAAAAAGQGGQGGYGRQSQGAGSAAAAAAAAAAAAAAGSGQGGYGGQGQGGYGQSSASASAAASAASTVANSVS

SEQ ID NO: 4 - protein, 23 aa, synthetic construct
  source 1..23: note = Consensus sequence derived from internal repeats of Euprosthenops australis MaSp1
  REGION 1..23: note = Consensus sequence derived from internal repeats of Euprosthenops australis MaSp1
  VARIANT 4: note = Ser
  VARIANT 8: note = Tyr
  VARIANT 11: note = Gln
GQGGQGGQGGLGQGGYGQGAGSS

SEQ ID NO: 5 - protein, 17 aa, synthetic construct
  source 1..17: note = Consensus sequence derived from internal repeats of Euprosthenops australis MaSp1
  REGION 1..17: note = Consensus sequence derived from internal repeats of Euprosthenops australis MaSp1
  VARIANT 9: note = Arg
  VARIANT 14: note = Ser
  VARIANT 16: note = Gly
GQGGQGQGGYGQGAGSS

SEQ ID NO: 6 - protein, 14 aa, synthetic construct
  source 1..14: note = Consensus sequence derived from internal repeats of Euprosthenops australis MaSp1
  REGION 1..14: note = Consensus sequence derived from internal repeats of Euprosthenops australis MaSp1
  VARIANT 2: note = Gln
  VARIANT 6: note = Arg
  VARIANT 11: note = Ser
  VARIANT 11: note = Val
GRGQGGYGQGAGGN

SEQ ID NO: 7 - protein, 18 aa, synthetic construct
  source 1..18: note = Consensus sequence
  REGION 1..18: note = Consensus sequence
ASASAAASAASTVANSVS

SEQ ID NO: 8 - protein, 8 aa, synthetic construct
  source 1..8: note = Consensus sequence
  REGION 1..8: note = Consensus sequence
ASAASAAA

SEQ ID NO: 9 - protein, 8 aa, synthetic construct
  source 1..8: note = Consensus sequence
  REGION 1..8: note = Consensus sequence
GSAMGQGS

SEQ ID NO: 10 - protein, 5 aa, synthetic construct
  source 1..5: note = Consensus sequence
  REGION 1..5: note = Consensus sequence
SASAG

SEQ ID NO: 11 - protein, 346 aa, synthetic construct
  source 1..346: note = Chimeric protein
  REGION 1..346: note = Chimeric protein
MGHHHHHHMSHTTPWTNPGLAENFMNSFMQGLSSMPGFTASQLDDMSTIAQSMVQSIQSLAAQGRTSPNKLQALNMAFASSMAEIAASEEGGGSLSTKTSSIASAMSNAFLQTTGVVNQPFINEITQLVSMFAQAGMNDVSAGNSGRGQGGYGQGSGGNAAAAAAAAAAAAAAAGQGGQGGYGRQSQGAGSAAAAAAAAAAAAAAGSGQGGYGGQGQGGYGQSGNSVTSGGYGYGTSAAAGAGVAAGSYAGAVNRLSSAEAASRVSSNIAAIASGGASALPSVISNIYSGVVASGVSSNEALIQALLELLSALVHVLSSASIGNVSSVGVDSTLNVVQDSVGQYVG

SEQ ID NO: 12 - DNA, 1052 bp, synthetic construct
  source 1..1052: mol_type = other DNA; note = Chimeric construct
  misc_feature 1..1052: note = Chimeric construct
ccatgggccatcatcatcatcatcatatgagccataccaccccgtggaccaacccgggcctggcggaaaactttatgaacagctttatgcagggcctgagcagcatgccgggctttaccgcgagccagctggatgatatgagcaccattgcgcagagcatggtgcagagcattcagagcctggcggcgcagggccgtaccagcccgaacaaactgcaggcgctgaacatggcgtttgcgagcagcatggcggaaattgcggcgagcgaagaaggcggcggcagcctgagcaccaaaaccagcagcattgcgagcgcgatgagcaacgcgtttctgcagaccaccggcgtggtgaaccagccgtttattaacgaaattacccagctggtgagcatgtttgcgcaggcgggcatgaacgatgtgagcgcggggaattcgggacgaggtcaaggaggatatggtcaaggttctggaggtaatgctgctgccgcagccgctgccgccgccgccgccgctgcagcagccggacagggaggtcaaggtggatatggtagacaaagccaaggtgctggttccgctgctgctgctgctgctgctgctgccgctgctgctgctgcaggatctggacaaggtggatacggtggacaaggtcaaggaggttatggtcagagtgggaattcggttacatctggaggttacggatatggaaccagtgcagctgcaggagctggagttgcagcaggttcatatgcaggtgctgtcaatcgcttgtctagtgctgaagctgccagtagagtatcctctaatattgcagctattgcatctggtggtgcttccgccctccccagtgttatttcaaatatttactcaggtgtcgttgcttctggtgtttcttctaatgaagctctgattcaagctctgttggaactcctttccgcacttgttcatgttttaagcagtgcctctatcggtaatgttagctcagtaggagtagatagtacattgaatgttgttcaggattcagtaggccaatatgtaggttaatgaaagctt

SEQ ID NO: 13 - DNA, 848 bp, synthetic construct
  source 1..848: mol_type = other DNA; note = Chimeric construct
  misc_feature 1..848: note = Chimeric construct
ccatgggccatcatcatcatcatcatatggggaattcgatgcagtacaaactgatcatcgacggtaaaaccctgaaaggtgaaaccaccaccgaagctgttgacgctgctgctgctgaaaaattcttcaaacagtacgctaacgacgacggtatcgacggtgaatggacctacgacgacgctaccaaaaccttcaccgttaccgaattagtacctagaggatcagggaattcgggacgaggtcaaggaggatatggtcaaggttctggaggtaatgctgctgccgcagccgctgccgccgccgccgccgctgcagcagccggacagggaggtcaaggtggatatggtagacaaagccaaggtgctggttccgctgctgctgctgctgctgctgctgccgctgctgctgctgcaggatctggacaaggtggatacggtggacaaggtcaaggaggttatggtcagagtgggaccggtgttacatctggaggttacggatatggaaccagtgcagctgcaggagctggagttgcagcaggtagttacgcaggtgctgtcaatcgcttgtctagtgctgaagctgccagtagagtatcctctaatattgcagctattgcatctggtggtgcttccgccctccccagtgttatttcaaatatttactcaggtgtcgttgcttctggtgtttcttctaatgaagctctgattcaagctctgttggaactcctttccgcacttgttcatgttttaagcagtgcctctatcggtaatgttagctcagtaggagtagatagtacattgaatgttgttcaggattcagtaggccaatatgtaggttaatgaaagctt

SEQ ID NO: 14 - protein, 278 aa, synthetic construct
  source 1..278: note = Chimeric protein
  REGION 1..278: note = Chimeric protein
MGHHHHHHMGNSMQYKLIIDGKTLKGETTTEAVDAAAAEKFFKQYANDDGIDGEWTYDDATKTFTVTELVPRGSGNSGRGQGGYGQGSGGNAAAAAAAAAAAAAAAGQGGQGGYGRQSQGAGSAAAAAAAAAAAAAAGSGQGGYGGQGQGGYGQSGTGVTSGGYGYGTSAAAGAGVAAGSYAGAVNRLSSAEAASRVSSNIAAIASGGASALPSVISNIYSGVVASGVSSNEALIQALLELLSALVHVLSSASIGNVSSVGVDSTLNVVQDSVGQYVG

SEQ ID NO: 15 - protein, 108 aa, Araneus ventricosus
AAGAGVAAGSYAGAVNRLSSAEAASRVSSNIAAIASGGASALPSVISNIYSGVVASGVSSNEALIQALLELLSALVHVLSSASIGNVSSVGVDSTLNVVQDSVGQYVG

SEQ ID NO: 16 - protein, 98 aa, Euprosthenops australis
SRLSSPSAVSRVSSAVSSLVSNGQVNMAALPNIISNISSSVSASAPGASGCEVIVQALLEVITALVQIVSSSSVGYINPSAVNQITNVVANAMAQVMG

SEQ ID NO: 17 - DNA, 1296 bp, synthetic construct
  source 1..1296: mol_type = other DNA; note = Chimeric construct
  misc_feature 1..1296: note = Chimeric construct
cccatgggccatcatcatcatcatcatatgagccataccaccccgtggaccaacccgggcctggcggaaaactttatgaacagctttatgcagggcctgagcagcatgccgggctttaccgcgagccagctggatgatatgagcaccattgcgcagagcatggtgcagagcattcagagcctggcggcgcagggccgtaccagcccgaacaaactgcaggcgctgaacatggcgtttgcgagcagcatggcggaaattgcggcgagcgaagaaggcggcggcagcctgagcaccaaaaccagcagcattgcgagcgcgatgagcaacgcgtttctgcagaccaccggcgtggtgaaccagccgtttattaacgaaattacccagctggtgagcatgtttgcgcaggcgggcatgaacgatgtgagcgcggggaattcgggacgaggtcaaggaggatatggtcaaggttctggaggtaatgctgctgccgcagccgctgccgccgccgccgccgctgcagcagccggacagggaggtcaaggtggatatggtagacaaagccaaggtgctggttccgctgctgctgctgctgctgctgctgccgctgctgctgctgcaggatctggacaaggtggatacggtggacaaggtcaaggaggttatggtcagagtgggaattcgggacgaggtcaaggaggatatggtcaaggttctggaggtaatgctgctgccgcagccgctgccgccgccgccgccgctgcagcagccggacagggaggtcaaggtggatatggtagacaaagccaaggtgctggttccgctgctgctgctgctgctgctgctgccgctgctgctgctgcaggatctggacaaggtggatacggtggacaaggtcaaggaggttatggtcagagtgggaattcggttacatctggaggttacggatatggaaccagtgcagctgcaggagctggagttgcagcaggttcatatgcaggtgctgtcaatcgcttgtctagtgctgaagctgccagtagagtatcctctaatattgcagctattgcatctggtggtgcttccgccctccccagtgttatttcaaatatttactcaggtgtcgttgcttctggtgtttcttctaatgaagctctgattcaagctctgttggaactcctttccgcacttgttcatgttttaagcagtgcctctatcggtaatgttagctcagtaggagtagatagtacattgaatgttgttcaggattcagtaggccaatatgtaggttaatgaaagctt

SEQ ID NO: 18 - protein, 427 aa, synthetic construct
  source 1..427: note = Chimeric sequence
  REGION 1..427: note = Chimeric sequence
MGHHHHHHMSHTTPWTNPGLAENFMNSFMQGLSSMPGFTASQLDDMSTIAQSMVQSIQSLAAQGRTSPNKLQALNMAFASSMAEIAASEEGGGSLSTKTSSIASAMSNAFLQTTGVVNQPFINEITQLVSMFAQAGMNDVSAGNSGRGQGGYGQGSGGNAAAAAAAAAAAAAAAGQGGQGGYGRQSQGAGSAAAAAAAAAAAAAAGSGQGGYGGQGQGGYGQSGNSGRGQGGYGQGSGGNAAAAAAAAAAAAAAAGQGGQGGYGRQSQGAGSAAAAAAAAAAAAAAGSGQGGYGGQGQGGYGQSGNSVTSGGYGYGTSAAAGAGVAAGSYAGAVNRLSSAEAASRVSSNIAAIASGGASALPSVISNIYSGVVASGVSSNEALIQALLELLSALVHVLSSASIGNVSSVGVDSTLNVVQDSVGQYVG

SEQ ID NO: 19 - protein, 97 aa, Parawixia bistriata
GAGAAAASGATGRVANSLGAMASGGINALPGVFSNIFSQVSAASGGASGGAVLVQALTEVIALLLHILSSASIGNVSSQGLEGSMAIAQQAIGAYAG

SEQ ID NO: 20 - protein, 88 aa, Tetragnatha kauaiensis
SLLSSPASNARISSAVSALASGAASGPGYLSSVISNVVSQVSSNSGGLVGCDTLVQALLEAAAALVHVLASSSGGQVNLNTAGYTSQL

SEQ ID NO: 21 - protein, 93 aa, Argiope trifasciata
AAASRLSSPQASSRVSSAVSTLVSSGPTNPASLSNAISSVVSQVSASNPGLSGCDVLVQALLEIVSALVHILGSSSIGQINYAASSQYAQMVG

SEQ ID NO: 22 - protein, 101 aa, Nephila clavipes
SAASRLSSPEASSRVSSAVSNLVSSGPTNSAALSSTISNVVSQIGASNPGLSGCDVLVQALLEVVSALIHILGSSSIGQVNYGSAGQATQIVGQSIYQALG

SEQ ID NO: 23 - protein, 101 aa, Nephila clavipes
AAASRLSSPQASSRVSSAVSNLVASGPTNSAALSSTISNVVSQIGASNPGLSGCDVLIQALLEVVSALIHILGSSSIGQVNYGSAGQATQIVGQSVYQALG

SEQ ID NO: 24 - protein, 101 aa, Latrodectus hesperus
AAASALAAPATSARISSHASALLSNGPTNPASISNVISNAVSQISSSNPGASACDVLVQALLELVTALLTIIGSSNIGSVNYDSSGQYAQVVTQSVQNAFA

SEQ ID NO: 25 - protein, 101 aa, Latrodectus hesperus
SAASALSSPTTHARISSHASTLLSSGPTNAAALSNVISNAVSQVSASNPGSSSCDVLVQALLEIITALISILDSSSVGQVNYGSSGQYAQIVGQSMQQAMG

SEQ ID NO: 26 - protein, 101 aa, Latrodectus geometricus
PAASALAAPATSARISSHALTLLSNGPTNPASISNVISNAVSQISSSNPGYSSCDILVQALLELVTALLTIIGSSNVNDINYGSSGQYAQMVSQSVQNVFG

SEQ ID NO: 27 - protein, 101 aa, Euprosthenops australis
NSVSRLSSPSAVSRVSSAVSSLVSNGQVNMAALPNIISNISSSVSASAPGASGCEVIVQALLEVITALVQIVSSSSVGYINPSAVNQITNVVANAMAQVMG

SEQ ID NO: 28 - protein, 98 aa, Nephila clavipes
PGSPGGAYYPSSRVPDMVNGIMSAMQGSGFNYQMFGNMLSQYSSGSGTCNPNNVNVLMDALLAALHCLSNHGSSSFAPSPTPAAMSAYSNSVGRMFAY

SEQ ID NO: 29 - protein, 98 aa, Nephila inaurata madagascariensis
GPGSGGSYYPSSRVPDMVNGIMSAMQGSGFNYQMFGNMLSQYSSGSGSCNPNNVNVLMDALLAALHCLSNHGSSSFAPSPTPAAMSAYSNSVGRMFAY

SEQ ID NO: 30 - protein, 93 aa, Latrodectus geometricus
SAASALSSPTTHARISSHASTLLSSGPTNSAAISNVISNAVSQVSASNPGSSSCDVLVQALLELITALISIVDSSNIGQVNYGSSGQYAQMVG

SEQ ID NO: 31 - protein, 101 aa, Latrodectus geometricus
AAASALAAPATSARISSHASTLLSNGPTNPASISNVISNAVSQISSSNPGASSCDVLVQALLELVTALLTIIGSSNVGNVNYDSSGQYAQVVSQSVQNAFV

SEQ ID NO: 32 - protein, 96 aa, Araneus diadematus
GAVNRLSSAGAASRVSSNVAAIASAGAAALPNVISNIYSGVLSSGVSSSEALIQALLEVISALIHVLGSASIGNVSSVGVNSALNAVQNAVGAYAG

SEQ ID NO: 33 - protein, 99 aa, Argiope trifasciata
SRLSSPGAASRVSSAVTSLVSSGGPTNSAALSNTISNVVSQISSSNPGLSGCDVLVQALLEIVSALVHILGSANIGQVNSSGVGRSASIVGQSINQAFS

SEQ ID NO: 34 - protein, 89 aa, Cyrtophora moluccensis
SHLSSPEASSRVSSAVSNLVSSGSTNSAALPNTISNVVSQISSSNPGLSGCDVLVQALLEVVSALIHILGSSSIGQVNYGSAGQATQIV

SEQ ID NO: 35 - protein, 87 aa, Nephila inaurata madagascariensis
SRLSSPQASSRVSSAVSNLVASGPTNSAALSSTISNAVSQIGASNPGLSGCDVLIQALLEVVSALIHILGSSSIGQVNYGSAGQATQ

SEQ ID NO: 36 - protein, 97 aa, Argiope amoena
RLSSPQASSRVSSAVSTLVSSGPTNPASLSNAIGSVVSQVSASNPGLPSCDVLVQALLEIVSALVHILGSSSIGQINYSASSQYARLVGQSIAQALG

SEQ ID NO: 37 - protein, 82 aa, Argiope aurantia
SRLSSPQASSRVSSAVSTLVSSGPTNPAALSNAISSVVSQVSASNPGLSGCDVLVQALLELVSALVHILGSSSIGQINYAAS

SEQ ID NO: 38 - protein, 98 aa, Argiope trifasciata
SRLSSPQASSRVSSAVSTLVSSGPTNPASLSNAISSVVSQVSSSNPGLSGCDVLVQALLEIVSALVHILGSSSIGQINYAASSQYAQLVGQSLTQALG

SEQ ID NO: 39 - protein, 89 aa, Gasteracantha mammosa
SRLSSPQAGARVSSAVSALVASGPTSPAAVSSAISNVASQISASNPGLSGCDVLVQALLEIVSALVSILSSASIGQINYGASGQYAAMI

SEQ ID NO: 40 - protein, 98 aa, Araneus diadematus
SRLSSPSAAARVSSAVSLVSNGGPTSPAALSSSISNVVSQISASNPGLSGCDILVQALLEIISALVHILGSANIGPVNSSSAGQSASIVGQSVYRALS

SEQ ID NO: 41 - protein, 98 aa, Araneus diadematus
SRLSSPAASSRVSSAVSSLVSSGPTKHAALSNTISSVVSQVSASNPGLSGCDVLVQALLEVVSALVSILGSSSIGQINYGASAQYTQMVGQSVAQALA

SEQ ID NO: 42 - protein, 100 aa, Deinopis spinosa
SAVSRMSTPGSGSRISNAVSNILSSGVSSSSGLSNAISNISSSISASNPGLSGCDVLVQVLLEVISALVHILGSASVGQVGSSPQNAQMVAANAVANAFS

SEQ ID NO: 43 - protein, 100 aa, Deinopis spinosa
SAVSRMSTPGSGSRISNAVSNILSSGVSSSSGLSNVISNLSSSISTSNPGLSGCDVLVQVLLEVISALVHILSSASLGQVGSSPQNAQMVAANAVANAFS

SEQ ID NO: 44 - protein, 96 aa, Metepeira grandiosa
GAVNRLSSAEAASRVSSNVAALASGGPAALANVMGNIYSGVASSGVSSGEALVQALLEVISALVHLLSNASIGNVSSAGLGNTMSLVQSTVGAYAG

SEQ ID NO: 45 - protein, 101 aa, Latrodectus hesperus
SAASRLSSPSSSSRISSAASSLATGGVLNSAALPSVVSNMMSQVSASSPGMSSSEVVIQALLELVSSLIHILSSANIGQVDFNSVGNTAAVVGQSLGAALG

SEQ ID NO: 46 - protein, 100 aa, Nephila clavipes
AAASRLASPDSGARVASAVSNLVSSGPTSSAALSSVISNAVSQIGASNPGLSGCDVLIQALLEIVSACVTILSSSSIGQVNYGAASQFAQVVGQSVLSAF

SEQ ID NO: 47 - protein, 85 aa, Nephila inaurata madagascariensis
AAASRLASPDSGARVASAVSNLVSSGPTSSAALSSVISNAVSQIGASNPGLSGCDVLIQALLEIVSACVTILSSSSIGQVNYGAA

SEQ ID NO: 48 - protein, 101 aa, Latrodectus hesperus
SAASRLSSPSSSSRISSAASSLATGGVLNSAALPSVVSNIMSQVSASSPGMSSSEVVIQALLELVSSLIHILSSANIGQVDFNSVGNTAAVVGQSLGAALG

SEQ ID NO: 49 - protein, 100 aa, synthetic construct
  source 1..100: note = Consensus sequence
  REGION 1..100: note = Consensus sequence
SRLSSPQASSRVSSAVSNLVSSGPTNSAALSNTISNVVSQISASNPGLSGCDVLVQALLEVVSALVHILGSSSIGQVNYGSAGQATQIVGQSVAQALGEF

SEQ ID NO: 50 - protein, 93 aa, Macrothele holsti
SHLSSPEASSRVSSAVSNLVSGGSTNSAALPNTISNVVSQISSSNPGLSGCDVLVQALLEVVSALIHILGSSSIGQVDYGSAGQATQIVGQSA

SEQ ID NO: 51 - protein, 89 aa, Nephila pilipes
SRLSSPEASSRVSSAVSNLVSSGPTNSAALSNTISNVVSQISSSNPGLSGCDVLVQALLEVVSALIHILGSSSIGQVNYGSAGQATQIV

SEQ ID NO: 52 - protein, 89 aa, Octonoba varians
SRLSSPEASSRVSSAVSNLVSSGPTNSAALSNTISNVVSQISSSNPGLSGCDVLVQALLEVVSAPIHILGSSSIGQVNYGSAGQATQIV

SEQ ID NO: 53 - protein, 89 aa, Psechrus sinensis
SRLSSPEASSRVSSAVSNLVSSGPTNSAALPNTISNVVSQISSSNPGLSGCDVLVQALLEVVSALIHILGSSSIGQVNYGSAGQATQIV

SEQ ID NO: 54 - protein, 88 aa, Tetragnatha versicolor
SRLSSPASNARISSAVSALASGGASSPGYLSSIISNVVSQVSSNNDGLSGCDTVVQALLEVAAALVHVLASSNIGQVNLNTAGYTSQL

SEQ ID NO: 55 - protein, 82 aa, Nephila senegalensis
  SITE 35: note = misc_feature - Xaa can be any naturally occurring amino acid
  SITE 56: note = misc_feature - Xaa can be any naturally occurring amino acid
SRLASPDSGARVASAVSNLVSSGPTSSAALSSVIXNAVSQIGASNPGLSGCDVLIXALLEIVSACVTILSSSSIGQVNYGAA

SEQ ID NO: 56 - protein, 94 aa, Araneus diadematus
SVYLRLQPRLEVSSAVSSLVSSGPTNGAAVSGALNSLVSQISASNPGLSGCDALVQALLELVSALVAILSSASIGQVNVSSVSQSTQMISQALS

SEQ ID NO: 57 - protein, 99 aa, Agelenopsis aperta
NSVSRLSSPSSSSRVSSAVSGLLPNGNFNLGNLPGIVSNLSSSIASSGLSGCENLVQVLIEVVSALVHILGSANIGNINMNAASSTAAAVGQAIVNGLY

SEQ ID NO: 58 - protein, 102 aa, Argiope argentata
ASSSGLGSSAASARVSSLANSVASAISSSGGSLSVPTFLNFLSSVGAQVSSSSSLNSSEVTNEVLLEAIAALLQVLNGAQITSVNLRNVPNAQQALVQALSG

SEQ ID NO: 59 - protein, 100 aa, synthetic construct
  source 1..100: note = Artificial construct
  REGION 1..100: note = Artificial construct
SRLSSPEASSRVSSAVSNLVSSGPTNSAALSSTISNVVSQIGASNPGLSGCDVLVQALLEVVSALIHILGSSSIGQVNYGSAGQATQLVGQSVYQALGEF

SEQ ID NO: 60 - protein, 87 aa, Nephila senegalensis
SRLSSPEASSRVSSAVSNLVSSGPTNSAALSSTISNVVSQIGASNPGLSGCDVLIQALLEVVSALVHILGSSSIGQVNYGSAGQATQ

SEQ ID NO: 61 - protein, 97 aa, Dolomedes tenebrosus
SRLSSPQAASRVSSAVSSLVSNGQVNVAALPSIISSLSSSISASSTAASDCEVLVQVLLEIVSALVQIVSSANVGYINPEASGSLNAVGSALAAAMG

SEQ ID NO: 62 - protein, 100 aa, Uloborus diversus
AASNRIVSAPAVNRMSAASSTLVSNGAFNVGALGSTISDMAAQIQAGSQGLSSAEATVQALLEVISVLTHMLSSANIGYVDFSRVGDSASAVSQSMAYAG

SEQ ID NO: 63 - protein, 102 aa, Argiope bruennichi
VSSSGLGSSAATARVSSLANSFASAISSSGGSLSVPTFLNLLSSVGAQVSSSSSLSSLEVTNEVLLEAIAALLQVINGGSITSVDLRYVPNAQQDLVNALSG

SEQ ID NO: 64 - protein, 96 aa, Araneus ventricosus
GAVNRLSSAEAASRVSSNIAAIASGGASALPSVISNIYSGVVASGVSSNEALIQALLELLSALVHVLSSASIGNVSSVGVDSTLNVVQDSVGQYVG

SEQ ID NO: 65 - protein, 101 aa, Nephila clavipes
STTSRLSSAEASSRISSAASTLVSGGYLNTAALPSVISDLFAQVGASSPGVSDSEVLIQVLLEIVSSLIHILSSSSVGQVDFSSVGSSAAAVGQSMQVVMG

SEQ ID NO: 66 - protein, 71 aa, Dolomedes tenebrosus
SRLSSPEAASRVSSAVSSLVSNGQVNVDALPSIISNLSSSISASATTASDCEVLVQVLLEVVSALVQIVCS

SEQ ID NO: 67 - protein, 102 aa, Agelenopsis aperta
SSETGLSSASASSRVNSLASSVASAIASGQALSADSFAKSLLIQASQIQSSAPSFKADDVVHESLLEGISALIQVINSSYGSPLSLSNAQTVNAGLVNYFLV

SEQ ID NO: 68 - protein, 102 aa, Nephila clavata
LSSSGLSSASASARVGSLAQSLASALSTSRGTLSLSTFLNLLSPISSEIRANTSLDGTQATVEALLEALAALLQVINGAQITDVNVSSVPSVNAALASALVA

SEQ ID NO: 69 - protein, 104 aa, Latrodectus hesperus
LSPAGLASTAATSRINDIAQSLSSTLSSGSQLAPDNVLPGLIQLSSSIQSGNPDLDPAGVLIESLLEYTSALLALLQNAQITTYDAATLPAFNTALVNYLVPLV

SEQ ID NO: 70 - protein, 95 aa, Argiope argentata
SVSRLSSAEAVSRVSSNIGAIASGGASALPGVISNIFSGVSASAGSYEEAVIQSLLEVLSALLHILSNSSIGYVGADGLTDSLAVVQQAMGPVVG

SEQ ID NO: 71 - protein, 101 aa, Nephila antipodiana
STTSRLSTAEASSRISTAASTLVSGGYLNTAALPSVIADLFAQVGASSPGVSDSEVLIQVLLEIVSSLIHILSSSSVGQVDFSSVGSSAAAVGQSMQVVMG

SEQ ID NO: 72 - protein, 100 aa, Nephila clavipes
STTSRLSSAEACSRISAAASTLVSGSLNTAALPSVISDLFAQVSASSPGVSGNEVLIQVLLEIVSSLIHILSSSSVGQVDFSSVGSSAAAVGQSMQVVMG

SEQ ID NO: 73 - protein, 103 aa, Deinopis spinosa
ASTSRLASGQATDRVKDVVSTLVSNGINGDALSNAISNVMTQVNAAVPGLSFCERLIQVLLEIVAALVHILSSSNVGSIDYGSTSRTAIGVSNALASAVAGAF

SEQ ID NO: 74 - protein, 352 aa, synthetic construct
  source 1..352: note = Artificial construct
  REGION 1..352: note = Artificial construct
MGHHHHHHMSHTTPWTNPGLAENFMNSFMQGLSSMPGFTASQLDDMSTIAQSMVQSIQSLAAQGRTSPNKLQALNMAFASSMAEIAASEEGGGSLSTKTSSIASAMSNAFLQTTGVVNQPFINEITQLVSMFAQAGMNDVSAGNSGRGQGGYGQGSGGNAAAAAAAAAAAAAAAGQGGQGGYGRQSQGAGSAAAAAAAAAAAAAAGSGQGGYGGQGQGGYGQSGSVTSGGYGYGTSAAAGAGVAAGSYAASTSRLASGQATDRVKDVVSTLVSNGINGDALSNAISNVMTQVNAAVPGLSFCERLIQVLLEIVAALVHILSSSNVGSIDYGSTSRTAIGVSNALASAVAGAF

SEQ ID NO: 75 - protein, 350 aa, synthetic construct
  source 1..350: note = Artificial construct
  REGION 1..350: note = Artificial construct
MGHHHHHHMSHTTPWTNPGLAENFMNSFMQGLSSMPGFTASQLDDMSTIAQSMVQSIQSLAAQGRTSPNKLQALNMAFASSMAEIAASEEGGGSLSTKTSSIASAMSNAFLQTTGVVNQPFINEITQLVSMFAQAGMNDVSAGNSGRGQGGYGQGSGGNAAAAAAAAAAAAAAAGQGGQGGYGRQSQGAGSAAAAAAAAAAAAAAGSGQGGYGGQGQGGYGQSGSVTSGGYGYGTSAAAGAGVAAGSYANSVSRLSSPSAVSRVSSAVSSLVSNGQVNMAALPNIISNISSSVSASAPGASGCEVIVQALLEVITALVQIVSSSSVGYINPSAVNQITNVVANAMAQVMG

SEQ ID NO: 76 - protein, 343 aa, synthetic construct
  source 1..343: note = Artificial construct
  REGION 1..343: note = Artificial construct
MGHHHHHHMSHTTPWTNPGLAENFMNSFMQGLSSMPGFTASQLDDMSTIAQSMVQSIQSLAAQGRTSPNKLQALNMAFASSMAEIAASEEGGGSLSTKTSSIASAMSNAFLQTTGVVNQPFINEITQLVSMFAQAGMNDVSAGNSGRGQGGYGQGSGGNAAAAAAAAAAAAAAAGQGGQGGYGRQSQGAGSAAAAAAAAAAAAAAGSGQGGYGGQGQGGYGQSGSVTSGGYGYGTSAAAGAGVAAGSYASVYLRLQPRLEVSSAVSSLVSSGPTNGAAVSGALNSLVSQISASNPGLSGCDALVQALLELVSALVAILSSASIGQVNVSSVSQSTQMISQALS

SEQ ID NO: 77 - protein, 350 aa, synthetic construct
  source 1..350: note = Artificial construct
  REGION 1..350: note = Artificial construct
MGHHHHHHMSHTTPWTNPGLAENFMNSFMQGLSSMPGFTASQLDDMSTIAQSMVQSIQSLAAQGRTSPNKLQALNMAFASSMAEIAASEEGGGSLSTKTSSIASAMSNAFLQTTGVVNQPFINEITQLVSMFAQAGMNDVSAGNSGRGQGGYGQGSGGNAAAAAAAAAAAAAAAGQGGQGGYGRQSQGAGSAAAAAAAAAAAAAAGSGQGGYGGQGQGGYGQSGSVTSGGYGYGTSAAAGAGVAAGSYASAASRLSSPSSSSRISSAASSLATGGVLNSAALPSVVSNMMSQVSASSPGMSSSEVVIQALLELVSSLIHILSSANIGQVDFNSVGNTAAVVGQSLGAALG

SEQ ID NO: 78 - protein, 346 aa, synthetic construct
  source 1..346: note = Artificial construct
  REGION 1..346: note = Artificial construct
MGHHHHHHMSHTTPWTNPGLAENFMNSFMQGLSSMPGFTASQLDDMSTIAQSMVQSIQSLAAQGRTSPNKLQALNMAFASSMAEIAASEEGGGSLSTKTSSIASAMSNAFLQTTGVVNQPFINEITQLVSMFAQAGMNDVSAGNSGRGQGGYGQGSGGNAAAAAAAAAAAAAAAGQGGQGGYGRQSQGAGSAAAAAAAAAAAAAAGSGQGGYGGQGQGGYGQSGNSVTSGGYGYGTSAAAGAGVAAGSYAGAVNRLSSAEAASAVSSNIAAIASGGASALPSVISNIYSGVVASGVSSNEALIQALLELLSALVHVLSSASIGNVSSVGVDSTLNVVQDSVGQYVG

SEQ ID NO: 79 - protein, 346 aa, synthetic construct
  source 1..346: note = Artificial construct
  REGION 1..346: note = Artificial construct
MGHHHHHHMSHTTPWTNPGLAENFMNSFMQGLSSMPGFTASQLDDMSTIAQSMVQSIQSLAAQGRTSPNKLQALNMAFASSMAEIAASEEGGGSLSTKTSSIASAMSNAFLQTTGVVNQPFINEITQLVSMFAQAGMNDVSAGNSGRGQGGYGQGSGGNAAAAAAAAAAAAAAAGQGGQGGYGRQSQGAGSAAAAAAAAAAAAAAGSGQGGYGGQGQGGYGQSGNSVTSGGYGYGTSAAAGAGVAAGSYAGAVNRLSSAEAASRVSSNIAAIASGGASALPSVISNIYSGVVASGVSSNEALIQALLELLSALVHVLSSASIGNVSSVGVASTLNVVQDSVGQYVG